European Patent Application EP 4 230 747 A2, published August 23, 2023. Title: COMPOSITIONS AND METHODS FOR NUCLEIC ACID SEQUENCING. Applicant: Pacific Biosciences of California, Inc. Application EP. The sequence listing filed with the application follows.

SEQUENCE LISTING (9 sequences)

SEQ ID NO: 1 - DNA, 35 bp, synthetic construct
  misc_feature 1..35: note = "Description of artificial sequence: Primer for amplification"
  source 1..35: mol_type = other DNA
gtacgggtctcacccggggatcctctagaatcgat

SEQ ID NO: 2 - DNA, 37 bp, synthetic construct
  misc_feature 1..37: note = "Description of artificial sequence: Primer for amplification"
  source 1..37: mol_type = other DNA
cctaaggtctcggaagctactagtcctcagcaagctt

SEQ ID NO: 3 - DNA, 24 bp, synthetic construct
  misc_feature 1..24: note = "Description of artificial sequence: Hairpin oligo"
  source 1..24: mol_type = other DNA
cgggctcggaacgaaagttccgag

SEQ ID NO: 4 - DNA, 74 bp, synthetic construct
  misc_feature 1..74: note = "Description of artificial sequence: Hairpin oligo"
  source 1..74: mol_type = other DNA
cttcggtcgccagattagaaaatcagtcacgtctagatgcagtcaggttcttaaatcctagttccttggcgacc

SEQ ID NO: 5 - DNA, 24 bp, synthetic construct
  misc_feature 1..24: note = "Description of artificial sequence: Sequencing primer"
  source 1..24: mol_type = other DNA
ctgactgcatctagacgtgactga

SEQ ID NO: 6 - DNA, 44 bp, synthetic construct
  misc_feature 1..44: note = "Description of artificial sequence: nucleic acid template"
  source 1..44: mol_type = other DNA
gaccgaagctgatgttaaacagtctatacgctttcacgggctcg

SEQ ID NO: 7 - DNA, 44 bp, synthetic construct
  misc_feature 1..44: note = "Description of artificial sequence: nucleic acid template"
  source 1..44: mol_type = other DNA
cgagcccgtgaaatcgtatagactgtttaacatcagcttcggtc

SEQ ID NO: 8 - DNA, 44 bp, synthetic construct
  misc_feature 1..44: note = "Description of artificial sequence: nucleic acid template"
  source 1..44: mol_type = other DNA
gaccgaagctgatgttaaacagtctatacgctatcacgggctcg

SEQ ID NO: 9 - DNA, 44 bp, synthetic construct
  misc_feature 1..44: note = "Description of artificial sequence: nucleic acid template"
  source 1..44: mol_type = other DNA
cgagcccgtgatatcgtatagactgtttaacatcagcttcggtc